European Patent Application EP 4 667 577 A1, published December 24, 2025. Title: ITR-Rep gene complex. Applicant: 株式会社シンプロジェン. Application JP. The sequence listing filed with the application follows.

SEQUENCE LISTING (40 sequences)

SEQ ID NO: 1 - DNA, 20 bp, synthetic construct
  source 1..20: mol_type = other DNA
catcaatgggcgtggatagc

SEQ ID NO: 2 - DNA, 24 bp, synthetic construct
  source 1..24: mol_type = other DNA
ggagttgttacgacattttggaaa

SEQ ID NO: 3 - DNA, 52 bp, synthetic construct
  source 1..52: mol_type = other DNA
ttagtaagcttccctcctgacgcggtaggaggaggggagggtgccctgcatg

SEQ ID NO: 4 - DNA, 56 bp, synthetic construct
  source 1..56: mol_type = other DNA
ccttttgctcacatgtcaattggtagatgtacctggacatccaggtgatgccggcg

SEQ ID NO: 5 - DNA, 60 bp, synthetic construct
  source 1..60: mol_type = other DNA
tgtacaggcgcgccgaattcgttttagggcggagtaacttgtatgtgttgggaattgtag

SEQ ID NO: 6 - DNA, 51 bp, synthetic construct
  source 1..51: mol_type = other DNA
agggaagcttactaaacggtacacaggaaacaggagacacaactccaagtg

SEQ ID NO: 7 - DNA, 76 bp, synthetic construct
  source 1..76: mol_type = other DNA
gaaaagtgccacctgacgtcgcggccgcgcgatcgcggtacccaactccatgctcaacagtccccaggtacagccc

SEQ ID NO: 8 - DNA, 60 bp, synthetic construct
  source 1..60: mol_type = other DNA
gaattcggcgcgcctgtacagcccgggcgaccgcaccctgtgacgaaagccgcccgcaag

SEQ ID NO: 9 - DNA, 74 bp, synthetic construct
  source 1..74: mol_type = other DNA
cgaaaagtgccacctaaataatgattttattttgactgatagtgacctgttcgttgcaacaaattgatgagcaa

SEQ ID NO: 10 - DNA, 73 bp, synthetic construct
  source 1..73: mol_type = other DNA
caggcccacctgctcagattacaacttttgtatacaaagttggcattataaaaaagcattgctcatcaatttg

SEQ ID NO: 11 - DNA, 34 bp, synthetic construct
  source 1..34: mol_type = other DNA
gcccgaatcccggccggccaccatggtgagcaag

SEQ ID NO: 12 - DNA, 34 bp, synthetic construct
  source 1..34: mol_type = other DNA
tgccacccgtggatccttacttgtacagctcgtc

SEQ ID NO: 13 - DNA, 35 bp, synthetic construct
  source 1..35: mol_type = other DNA
ataaagttggcggccgctcgcgaagcgcctcccac

SEQ ID NO: 14 - DNA, 35 bp, synthetic construct
  source 1..35: mol_type = other DNA
agccatacctgatttaaatcatttattgctcagaa

SEQ ID NO: 15 - DNA, 108 bp, synthetic construct
  source 1..108: mol_type = other DNA
gaaaagtgccacctgacgtcgcggccgcggaggggtggagtcgtgacgtgaattacgtcatagggttagggaggtcctgtattagaggtcacgtgagtgttttgcgac

SEQ ID NO: 16 - DNA, 99 bp, synthetic construct
  source 1..99: mol_type = other DNA
gttcaaacctcccgcttcaaaatggagaccctgcgtgctcactcgggcttaaatacccagcgtgaccacatggtgtcgcaaaatgtcgcaaaacactca

SEQ ID NO: 17 - DNA, 41 bp, synthetic construct
  source 1..41: mol_type = other DNA
gcgggaggtttgaacgcgcagccgccatgccggggttttac

SEQ ID NO: 18 - DNA, 38 bp, synthetic construct
  source 1..38: mol_type = other DNA
actagtagcgctatttaaatcatttattgttcaaagat

SEQ ID NO: 19 - DNA, 32 bp, synthetic construct
  source 1..32: mol_type = other DNA
aatagcgctgcgatcgcggcctccaaaaaagc

SEQ ID NO: 20 - DNA, 37 bp, synthetic construct
  source 1..37: mol_type = other DNA
ccttttgctcacatgtcaattgatcccgcccctaact

SEQ ID NO: 21 - DNA, 23 bp, synthetic construct
  source 1..23: mol_type = other DNA
aacaataaatgatttaaatcagg

SEQ ID NO: 22 - DNA, 38 bp, synthetic construct
  source 1..38: mol_type = other DNA
ggccgcgatcgcagcgctgtagccatggaaactagata

SEQ ID NO: 23 - DNA, 75 bp, synthetic construct
  source 1..75: mol_type = other DNA
gtgccacctgacgtcaaataatgattttattttgactgatagtgacctgttcgttgcaacaaattgatgagcaat

SEQ ID NO: 24 - DNA, 74 bp, synthetic construct
  source 1..74: mol_type = other DNA
cgactccacccctccgcggccgccaactttattatacaaagttggcattataaaaaagcattgctcatcaattt

SEQ ID NO: 25 - DNA, 78 bp, synthetic construct
  source 1..78: mol_type = other DNA
catggctacagcgctgcgatcgcacccagctttcttgtacaaagttggcattataagaaagcattgcttatcaatttg

SEQ ID NO: 26 - DNA, 75 bp, synthetic construct
  source 1..75: mol_type = other DNA
tttttggaggccgcgcaaataatgattttattttgactgatagtgacctgttcgttgcaacaaattgataagcaa

SEQ ID NO: 27 - DNA, 35 bp, synthetic construct
  source 1..35: mol_type = other DNA
ataaagttggcggccgcagtgacgtaacgcgaagc

SEQ ID NO: 28 - DNA, 35 bp, synthetic construct; identical to SEQ ID NO: 14
  source 1..35: mol_type = other DNA

SEQ ID NO: 29 - DNA, 35 bp, synthetic construct
  source 1..35: mol_type = other DNA
ataaagttggcggccgcgggttttgtaagcagtga

SEQ ID NO: 30 - DNA, 35 bp, synthetic construct
  source 1..35: mol_type = other DNA
agccatacctgatttaaatcatttactgttcttta

SEQ ID NO: 31 - DNA, 34 bp, synthetic construct
  source 1..34: mol_type = other DNA
ataaagttggcggccgcaagcgcctcccacgctg

SEQ ID NO: 32 - DNA, 35 bp, synthetic construct; identical to SEQ ID NO: 14
  source 1..35: mol_type = other DNA

SEQ ID NO: 33 - DNA, 35 bp, synthetic construct
  source 1..35: mol_type = other DNA
ataaagttggcggccgccagagagggagtggccaa

SEQ ID NO: 34 - DNA, 35 bp, synthetic construct; identical to SEQ ID NO: 14
  source 1..35: mol_type = other DNA

SEQ ID NO: 35 - DNA, 35 bp, synthetic construct; identical to SEQ ID NO: 33
  source 1..35: mol_type = other DNA

SEQ ID NO: 36 - DNA, 35 bp, synthetic construct; identical to SEQ ID NO: 14
  source 1..35: mol_type = other DNA

SEQ ID NO: 37 - DNA, 23 bp, synthetic construct
  source 1..23: mol_type = other DNA
aacaataaatgatttaaatcagg

SEQ ID NO: 38 - DNA, 38 bp, synthetic construct; identical to SEQ ID NO: 22
  source 1..38: mol_type = other DNA

SEQ ID NO: 39 - DNA, 20 bp, synthetic construct
  source 1..20: mol_type = other DNA
catcaatgggcgtggatagc

SEQ ID NO: 40 - DNA, 24 bp, synthetic construct
  source 1..24: mol_type = other DNA
ggagttgttacgacattttggaaa